European Patent Application EP 4 538 281 A1, published April 16, 2025. Title: Peptide having activities of muscle loss inhibition and muscle mass enhancement and uses thereof. Applicant: CAREGEN CO., LTD. Application KR. The sequence listing filed with the application follows.

SEQUENCE LISTING (1 sequence)

SEQ ID NO: 1 - protein, 7 aa, synthetic construct
EAEYEHL